European Patent Application EP 4 640 232 A1, published October 29, 2025. Title: 一种重组蛋白用于制备抑制动脉瘤药物的应用. Applicant: 华中科技大学. The sequence listing filed with the application follows.

SEQUENCE LISTING (4 sequences)

SEQ ID NO: 1 - protein, 714 aa, human
MASEAPSPPRSPPPPTSPEPELAQLRRKVEKLERELRSCKRQVREIEKLLHHTERLYQNAESNNQELRTQVEELSKILQRGRNEDNKKSDVEVQTENHAPWSISDYFYQTYYNDVSLPNKVTELSDQQDQAIETSILNSKDHLQVENDAYPGTDRTENVKYRQVDHFASNSQEPASALATEDTSLEGSSLAESLRAAAEAAVSQTGFSYDENTGLYFDHSTGFYYDSENQLYYDPSTGIYYYCDVESGRYQFHSRVDLQPYPTSSTKQSKDKKLKKKRKDPDSSATNEEKDLNSEDQKAFSVEHTSCNEEENFANMKKKAKIGIHHKNSPPKVTVPTSGNTIESPLHENISNSTSFKDEKIMETDSEPEEGEITDSQTEDSYDEAITSEGNVTAEDSEDEDEDKIWPPCIRVIVIRSPVLQIGSLFIITAVNPATIGREKDMEHTLRIPEVGVSKFHAEIYFDHDLQSYVLVDQGSQNGTIVNGKQILQPKTKCDPYVLEHGDEVKIGETVLSFHIHPGSDTCDGCEPGQVRAHLRLDKKDESFVGPTLSKEEKELERRKELKKIRVKYGLQNTEYEDEKTLKNPKYKDRAGKRREQVGSEGTFQRDDAPASVHSEITDSNKGRKMLEKMGWKKGEGLGKDGGGMKTPIQLQLRRTHAGLGTGKPSSFEDVHLLQNKNKKNWDKARERFTENFPETKPQKDDPGTMPWVKGTLE

SEQ ID NO: 2 - DNA, 2145 bp, human
  source 1..2145: mol_type = genomic DNA
atggcctcggaggcgccgtccccgccgcggtcgccgccgccgcccacctcccccgagcctgagctggcccagctaaggcggaaggtggagaagttggaacgtgaactgcggagctgcaagcggcaggtgcgggagatcgagaagctgctgcatcacacagaacggctgtaccagaacgcagaaagcaacaaccaggagctccgcacgcaggtggaagaactcagtaaaatactccaacgtgggagaaatgaagataataaaaagtctgatgtagaagtacaaacagagaaccatgctccttggtcaatctcagattatttttatcagacgtactacaatgacgttagtcttccaaataaagtgactgaactgtcagatcaacaagatcaagctatcgaaacttctattttgaattctaaagaccatttacaagtagaaaatgatgcttaccctggtaccgatagaacagaaaatgttaaatatagacaagtggaccattttgcctcaaattcacaggagccagcatctgcattagcaacagaagatacctccttagaaggctcatcattagctgaaagtttgagagctgcagcagaagcggctgtatcacagactggatttagttatgatgaaaatactggactgtattttgaccacagcactggtttctattatgattctgaaaatcaactctattatgatccttccactggaatttattactattgtgatgtggaaagtggtcgttatcagtttcattctcgagtagatttgcaaccttatccgacttctagcacaaaacaaagtaaagataaaaaattgaagaagaaaagaaaagatccagattcttctgcaacaaatgaggaaaaggatttgaactcagaggatcaaaaagccttcagtgttgaacatacaagctgcaatgaggaagaaaatttcgcaaatatgaaaaagaaggccaaaataggcattcatcacaaaaatagtccccccaaagtcactgttccaactagtggaaatactatagagtctcctcttcatgaaaacatctctaattcaacatcatttaaagatgagaaaatcatggagactgatagtgaaccagaggaaggtgaaattacagactctcagactgaggatagttatgacgaagccattaccagtgaaggcaatgtaactgcagaagatagtgaggatgaagatgaagacaaaatttggcccccatgtattagagtaattgtcattagatcacctgtgttgcagataggatcactctttatcattactgctgtaaaccctgctacaattggaagagaaaaggatatggaacatactctccgaatccctgaagttggtgtcagtaagtttcatgcagaaatttattttgaccatgacttacaaagttatgtccttgtggatcaaggcagtcaaaatggcacaattgttaatggaaaacagattcttcagccgaaaactaaatgtgacccttacgtacttgagcatggagatgaagtcaaaattggagaaactgtcttatcctttcacattcatcctggcagtgatacctgtgatggctgtgaaccagggcaggttagagcccaccttcgccttgataagaaagatgaatcttttgttggtccaacactaagtaaggaggaaaaagagttggaaagaagaaaagaattaaagaaaatacgagtaaaatatggtttacagaatacagaatacgaagatgaaaagacattgaagaatccaaaatataaagatagagctggaaaacgtagggagcaggttggaagtgaaggaactttccaaagagatgatgctcctgcatctgttcattctgaaattactgatagcaacaaaggtcggaagatgttggagaagatgggttggaagaaaggagagggcctggggaaggatggtggaggaatgaaaacgccgatccagcttcagcttcggcgaacacatgcaggcttggggacaggcaaaccatcctcatttgaagatgttcaccttctccaaaacaagaacaaaaaaaactgggacaaagcacgagagcggtttactgaaaacttcccagaaactaagcctcaaaaagatgacccagggaccatgccttgggtaaaagggactttagagtga

SEQ ID NO: 3 - DNA, 32 bp, synthetic construct
  source 1..32: mol_type = other DNA
gcggatccatggcctcggaggcgccgtccccg

SEQ ID NO: 4 - DNA, 32 bp, synthetic construct
  source 1..32: mol_type = other DNA
ccaagctttcactctaaagtcccttttaccca